European Patent Application EP 4 130 039 A1, published February 8, 2023. Title: DEVELOPMENT AND APPLICATION OF IMMUNE CELL ACTIVATOR. Applicant: BIO-THERA SOLUTIONS, LTD. Application EP 21 775 350.8. The sequence listing filed with the application follows.

SEQUENCE LISTING (106 sequences)

SEQ ID NO: 1 - protein, 8 aa, Artificial Sequence
GFTFSSYA

SEQ ID NO: 2 - protein, 8 aa, Artificial Sequence
ISYDGSNK

SEQ ID NO: 3 - protein, 16 aa, Artificial Sequence
ARELGVYSGYDTPFDY

SEQ ID NO: 4 - protein, 8 aa, Artificial Sequence
GFTFDDYA

SEQ ID NO: 5 - protein, 8 aa, Artificial Sequence
IGGSGGST

SEQ ID NO: 6 - protein, 15 aa, Artificial Sequence
AKDRGYGDYYWYFDL

SEQ ID NO: 7 - protein, 17 aa, Artificial Sequence
VISEDGSNQYYADSVKG

SEQ ID NO: 8 - protein, 8 aa, Artificial Sequence
ISGSGGNT

SEQ ID NO: 9 - protein, 15 aa, Artificial Sequence
AKDPLGSSWFEYFQH

SEQ ID NO: 10 - protein, 5 aa, Artificial Sequence
SYGMH

SEQ ID NO: 11 - protein, 17 aa, Artificial Sequence
VISYDGSNQYYADSVKG

SEQ ID NO: 12 - protein, 13 aa, Artificial Sequence
DNQDSSPDVGIDY

SEQ ID NO: 13 - protein, 17 aa, Artificial Sequence
VIAEVGSNQYYADSVKG

SEQ ID NO: 14 - protein, 8 aa, Artificial Sequence
ISNSGGST

SEQ ID NO: 15 - protein, 9 aa, Artificial Sequence
AKDGPYFDY

SEQ ID NO: 16 - protein, 8 aa, Artificial Sequence
GFTFSTYA

SEQ ID NO: 17 - protein, 8 aa, Artificial Sequence
ISGTGDWA

SEQ ID NO: 18 - protein, 17 aa, Artificial Sequence
AKSSSTVATDFDYGMDV

SEQ ID NO: 19 - protein, 7 aa, Artificial Sequence
AAVALQS

SEQ ID NO: 20 - protein, 8 aa, Artificial Sequence
ISGSGGST

SEQ ID NO: 21 - protein, 13 aa, Artificial Sequence
ARGDSSSWFIFQD

SEQ ID NO: 22 - protein, 8 aa, Artificial Sequence
GFTVSSNY

SEQ ID NO: 23 - protein, 7 aa, Artificial Sequence
IYYGGST

SEQ ID NO: 24 - protein, 11 aa, Artificial Sequence
ARVVVPGYFDL

SEQ ID NO: 25 - protein, 7 aa, Artificial Sequence
AAVGLQS

SEQ ID NO: 26 - protein, 17 aa, Artificial Sequence
VIWEDGSNQYYADSVKG

SEQ ID NO: 27 - protein, 13 aa, Artificial Sequence
DNQDTSPDVGIDY

SEQ ID NO: 28 - protein, 6 aa, Artificial Sequence
RDIRDD

SEQ ID NO: 29 - protein, 3 aa, Artificial Sequence
AAS

SEQ ID NO: 30 - protein, 9 aa, Artificial Sequence
LQDSDYPLT

SEQ ID NO: 31 - protein, 9 aa, Artificial Sequence
SSDVGGYNY

SEQ ID NO: 32 - protein, 3 aa, Artificial Sequence
DVS

SEQ ID NO: 33 - protein, 10 aa, Artificial Sequence
SSYTTSSTLV

SEQ ID NO: 34 - protein, 9 aa, Artificial Sequence
QQYTDYPLT

SEQ ID NO: 35 - protein, 3 aa, Artificial Sequence
EVS

SEQ ID NO: 36 - protein, 11 aa, Artificial Sequence
SSYSSSSTLVV

SEQ ID NO: 37 - protein, 6 aa, Artificial Sequence
QDILGY

SEQ ID NO: 38 - protein, 3 aa, Artificial Sequence
ATS

SEQ ID NO: 39 - protein, 9 aa, Artificial Sequence
QQYNSYPLT

SEQ ID NO: 40 - protein, 8 aa, Artificial Sequence
QSISSYLN

SEQ ID NO: 41 - protein, 9 aa, Artificial Sequence
QQYDDYPLT

SEQ ID NO: 42 - protein, 9 aa, Artificial Sequence
LQIDSYPLT

SEQ ID NO: 43 - protein, 11 aa, Artificial Sequence
RASQNISPFLN

SEQ ID NO: 44 - protein, 7 aa, Artificial Sequence
AASSLQS

SEQ ID NO: 45 - protein, 9 aa, Artificial Sequence
QQYNDYPLT

SEQ ID NO: 46 - protein, 6 aa, Artificial Sequence
QGIGDD

SEQ ID NO: 47 - protein, 3 aa, Artificial Sequence
KAS

SEQ ID NO: 48 - protein, 9 aa, Artificial Sequence
QQAHSFPPT

SEQ ID NO: 49 - protein, 9 aa, Artificial Sequence
EEIGSWLAW

SEQ ID NO: 50 - protein, 3 aa, Artificial Sequence
EAS

SEQ ID NO: 51 - protein, 9 aa, Artificial Sequence
QQYGSYPPT

SEQ ID NO: 52 - protein, 6 aa, Artificial Sequence
EDIGRW

SEQ ID NO: 53 - protein, 9 aa, Artificial Sequence
QQYSDYPLT

SEQ ID NO: 54 - protein, 9 aa, Artificial Sequence
QQYYNYPPT

SEQ ID NO: 55 - protein, 8 aa, Artificial Sequence
SSNMGSNP

SEQ ID NO: 56 - protein, 3 aa, Artificial Sequence
NNN

SEQ ID NO: 57 - protein, 11 aa, Artificial Sequence
AAWDDGLNGWV

SEQ ID NO: 58 - protein, 9 aa, Artificial Sequence
DSLRSYYAS

SEQ ID NO: 59 - protein, 3 aa, Artificial Sequence
NNR

SEQ ID NO: 60 - protein, 10 aa, Artificial Sequence
HSRDSSGKYV

SEQ ID NO: 61 - protein, 11 aa, Artificial Sequence
RASQNISPFLN

SEQ ID NO: 62 - protein, 7 aa, Artificial Sequence
AAVGSQS

SEQ ID NO: 63 - protein, 8 aa, Artificial Sequence
QQYTDYPL

SEQ ID NO: 64 - protein, 123 aa, Artificial Sequence
QVQLQESGGGLEKPGRSLRLSCAASGFTFSSYAMHWVRQAPGKGLEWVAVISYDGSNKYYADSVKGRFTISRDNSKNTLYLQMNSLRAEDTAVYYCARELGVYSGYDTPFDYWGQGTLVTVSS

SEQ ID NO: 65 - protein, 122 aa, Artificial Sequence
EVQLVESGGGLVQPGRSLRLSCAASGFTFDDYAMHWVRQAPGRGLEWVSGIGGSGGSTYYADSVKGRFTISRDNSKNTLYLQMNGLGAEDTAVYYCAKDRGYGDYYWYFDLWGRGTLVTVSS

SEQ ID NO: 66 - protein, 122 aa, Artificial Sequence
QVQLRESGGGLVQPGGSLRLSCAASGFTFSSYAMNWVRQAPGKGLEWVSAISGSGGNTYYADSVKGRLTISRDNSKNTLYLQMNSLRAEDTAVYYCAKDPLGSSWFEYFQHWGQGTLVTVSS

SEQ ID NO: 67 - protein, 122 aa, Artificial Sequence
QVQLEESGGGVVQPGESLRLSCAASGFTFSSYGMHWVRQAPGKGLEWVAVISYDGSNQYYADSVKGRFTISRDNSKNTLYLQMNSLRAEDTAVYYCAKDNQDSSPDVGIDYWGQGTLVTVSS

SEQ ID NO: 68 - protein, 116 aa, Artificial Sequence
QVQLQRSGGGLVQPGGSLRLSCAASGFTFSSYGMTWVRQAPGKGLEWVSAISNSGGSTYYADSVKGRFTISRDNSKNTLYLQMNSLRAEDTAVYYCAKDGPYFDYWGQGTLVTVSS

SEQ ID NO: 69 - protein, 124 aa, Artificial Sequence
QVQLVESGGGLIQPGGSLRLSCTASGFTFSTYAMSWVRQAPGKGLEWVSAISGTGDWASYADSVKGRFTTSRDNSRNTLYLQMNNLRDEDTAIYYCAKSSSTVATDFDYGMDVWGQGTLVTVSS

SEQ ID NO: 70 - protein, 120 aa, Artificial Sequence
QVQLVESGGGLVQPGGSLRLSCAASGFTFSSYAMSWVRQAPGKGLEWVSAISGSGGSTYYADSVKGRFTISRDNSKNSLYLQMNSLRAEDTAVYYCARGDSSSWFIFQDWGQGTLVTVSS

SEQ ID NO: 71 - protein, 117 aa, Artificial Sequence
QVQLVESGGGLIQPGGSLRLSCAASGFTVSSNYMSWVRQAPGEGLEWIATIYYGGSTYYNPSLKSRVTISADMSKNQFSLKLSSMTAADTAVYYCARVVVPGYFDLWGRGTLVTVSS

SEQ ID NO: 72 - protein, 122 aa, Artificial Sequence
QVQLVESGGGVVQPGESLRLSCAASGFTFSSYGMHWVRQAPGKGLEWVAVIWEDGSNQYYADSVKGRFTISRDNSKNTLYLQMNSLRAEDTAVYYCAKDNQDTSPDVGIDYWGQGTLVTVSS

SEQ ID NO: 73 - protein, 107 aa, Artificial Sequence
DIQMTQSPSSLSASVGDRITITCRASRDIRDDLAWYQQKPGGAPKLLIYAASTLQSGVPSRFSGSGSGTDFTLTISSLQPEDFATYYCLQDSDYPLTFGGGTKLEIK

SEQ ID NO: 74 - protein, 110 aa, Artificial Sequence
SSELTQPASVSGSPGQSITISCTGTSSDVGGYNYVSWYQQHPGKAPKLMIYDVSNRPSGVSNRFSGSKSGNTASLTISGLQAEDEADYYCSSYTTSSTLVFGGGTKVTVL

SEQ ID NO: 75 - protein, 111 aa, Artificial Sequence
QSALTQPASVSGSPGQSITISCTGTSSDVGGYNYVSWYQKHPGKAPKLMIYEVSNRPSGVSNRFSGSKSANTASLTISGLQAEDEADYFCSSYSSSSTLVVFGGGTKLTVL

SEQ ID NO: 76 - protein, 107 aa, Artificial Sequence
DIVMTQSPSSLSASVGDRVTITCRASQDILGYVNWYQQKPGKAPILLIYATSGLQGGVPSRFSGSGSGTDFTLTISSLQPEDFATYYCQQYNSYPLTFGGGTKVDIK

SEQ ID NO: 77 - protein, 107 aa, Artificial Sequence
DIQMTQSPSSLSASVGDRVTITCRASQSISSYLNWYQQKPGKAPKLLMYAASSLQSGVPSRFSGSGSGTDFTLTISSLQPEDFATYYCLQIDSYPLTFGGGTKVEIK

SEQ ID NO: 78 - protein, 107 aa, Artificial Sequence
DIQMTQSPSSLSASVGDTVTITCRASQNISPFLNWYQQKPGKAPKLLIYAASSLQSGVPSRFSGSGSGTDFTLTISSLQPEDFATYYCQQYNSYPLTFGGGTKVEIK

SEQ ID NO: 79 - protein, 107 aa, Artificial Sequence
DIQMTQSPSTLSASVGDRVTITCRVSQGIGDDLGWYQQKPGKAPKLLIYKASNLESGVPSRFSGSGSGTDFSLTISSLQPEDFATYFCQQAHSFPPTFGGGTKLEIK

SEQ ID NO: 80 - protein, 107 aa, Artificial Sequence
ETTLTQSPSTLSASVGDRVTITCRASEEIGSWLAWYQQTPGKAPKRLIYEASSLQSGVPSRFSGSGSGTDFTLTISSLQPEDFATYYCQQYGSYPPTFGQGTKVEIK

SEQ ID NO: 81 - protein, 107 aa, Artificial Sequence
DIVMTQSPSTLSASVGDRVTVTCRASEDIGRWLAWYQQKPGKAPKRLIYAASSLQSGVPSRFSGSGSGTEFTLTISSLQPEDFATYYCQQYYNYPPTFGQGTKVEIK

SEQ ID NO: 82 - protein, 110 aa, Artificial Sequence
QSVLTQPPSASGTPGQRVTISCSGSSSNMGSNPVNWYQQLPGEAPQLLMYNNNQRPSGVPDRFSGSKSGTSASLAISGLQSEDEAEYYCAAWDDGLNGWVFGGGTKLTVL

SEQ ID NO: 83 - protein, 107 aa, Artificial Sequence
SSELTQDPAVSVALGQTVSITCQGDSLRSYYASWYQQKPGQAPVPVIYGKNNRPSGIPDRFSGSSSGNTASLTITGAQAEDEADYYCHSRDSSGKYVFGVGTKLTVL

SEQ ID NO: 84 - protein, 107 aa, Artificial Sequence
DIQMTQSPSSLSASVGDRVTITCRASQNISPFLNWYQQKPGKAPKLLIYAAVGLQSGVPSRFSGSGSGTDFTLTISSLQPEDFATYYCQQYTDYPLTFGGGTKVEIK

SEQ ID NO: 85 - protein, 19 aa, Artificial Sequence
MEFGLSWVFLVAILKGVQC

SEQ ID NO: 86 - protein, 452 aa, Artificial Sequence
QVQLVESGGGVVQPGESLRLSCAASGFTFSSYGMHWVRQAPGKGLEWVAVIWEDGSNQYYADSVKGRFTISRDNSKNTLYLQMNSLRAEDTAVYYCAKDNQDTSPDVGIDYWGQGTLVTVSSASTKGPSVFPLAPSSKSTSGGTAALGCLVKDYFPEPVTVSWNSGALTSGVHTFPAVLQSSGLYSLSSVVTVPSSSLGTQTYICNVNHKPSNTKVDKKVEPKSCDKTHTCPPCPAPELLGGPSVFLFPPKPKDTLMISRTPEVTCVVVDVSHEDPEVKFNWYVDGVEVHNAKTKPREEQYNSTYRVVSVLTVLHQDWLNGKEYKCKVSNKALPAPIEKTISKAKGQPREPQVYTLPPSRDELTKNQVSLTCLVKGFYPSDIAVEWESNGQPENNYKTTPPVLDSDGSFFLYSKLTVDKSRWQQGNVFSCSVMHEALHNHYTQKSLSLSPGK

SEQ ID NO: 87 - protein, 214 aa, Artificial Sequence
DIQMTQSPSSLSASVGDRVTITCRASQNISPFLNWYQQKPGKAPKLLIYAAVGLQSGVPSRFSGSGSGTDFTLTISSLQPEDFATYYCQQYTDYPLTFGGGTKVEIKRTVAAPSVFIFPPSDEQLKSGTASVVCLLNNFYPREAKVQWKVDNALQSGNSQESVTEQDSKDSTYSLSSTLTLSKADYEKHKVYACEVTHQGLSSPVTKSFNRGEC

SEQ ID NO: 88 - protein, 330 aa, Artificial Sequence
ASTKGPSVFPLAPSSKSTSGGTAALGCLVKDYFPEPVTVSWNSGALTSGVHTFPAVLQSSGLYSLSSVVTVPSSSLGTQTYICNVNHKPSNTKVDKKVEPKSCDKTHTCPPCPAPELLGGPSVFLFPPKPKDTLMISRTPEVTCVVVDVSHEDPEVKFNWYVDGVEVHNAKTKPREEQYNSTYRVVSVLTVLHQDWLNGKEYKCKVSNKALPAPIEKTISKAKGQPRRPQVYTLPPSRDELTKNQVSLTCLVKGFYPSDIAVEWESNGQPENNYKTTPPVLDSDGSFFLYSKLTVDKSRWQQGNVFSCSVMHEALHNHYTQKYLSLSPGK

SEQ ID NO: 89 - protein, 330 aa, Artificial Sequence
ASTKGPSVFPLAPSSKSTSGGTAALGCLVKDYFPEPVTVSWNSGALTSGVHTFPAVLQSSGLYSLSSVVTVPSSSLGTQTYICNVNHKPSNTKVDKKVEPKSCDKTHTCPPCPAPELLGGPSVFLFPPKPKDTLMISRTPEVTCVVVDVSHEDPEVKFNWYVDGVEVHNAKTKPREEQYNSTYRVVSVLTVLHQDWLNGKEYKCKVSNKALPAPIEKTISKAKGQPRRPQVYTLPPSRDELTKNQVSLTCLVKGFYPSDIAVEWESNGQPENNYKTTPPVLDSDGSFFLYSKLTVDKSRWQQGNVFSCSVMHEALHNHYTQKSLSLSPGK

SEQ ID NO: 90 - protein, 330 aa, Artificial Sequence [sequence omitted]

SEQ ID NO: 91 - protein, 107 aa, Artificial Sequence [sequence omitted]

SEQ ID NO: 92 - protein, 326 aa, Artificial Sequence
ASTKGPSVFPLAPCSRSTSESTAALGCLVKDYFPEPVTVSWNSGALTSGVHTFPAVLQSSGLYSLSSVVTVPSSNFGTQTYTCNVDHKPSNTKVDKTVERKCCVECPPCPAPPVAGPSVFLFPPKPKDTLMISRTPEVTCVVVDVSHEDPEVQFNWYVDGVEVHNAKTKPREEQFNSTFRVVSVLTVVHQDWLNGKEYKCKVSNKGLPAPIEKTISKTKGQPREPQVYTLPPSREEMTKNQVSLTCLVKGFYPSDIAVEWESNGQPENNYKTTPPMLDSDGSFFLYSKLTVDKSRWQQGNVFSCSVMHEALHNHYTQKSLSLSPGK

SEQ ID NO: 93 - protein, 107 aa, Artificial Sequence [sequence omitted]

SEQ ID NO: 94 - protein, 327 aa, Artificial Sequence
ASTKGPSVFPLAPCSRSTSESTAALGCLVKDYFPEPVTVSWNSGALTSGVHTFPAVLQSSGLYSLSSVVTVPSSSLGTKTYTCNVDHKPSNTKVDKRVESKYGPPCPPCPAPEFLGGPSVFLFPPKPKDTLMISRTPEVTCVVVDVSQEDPEVQFNWYVDGVEVHNAKTKPREEQFNSTYRVVSVLTVLHQDWLNGKEYKCKVSNKGLPSSIEKTISKAKGQPREPQVYTLPPSQEEMTKNQVSLTCLVKGFYPSDIAVEWESNGQPENNYKTTPPVLDSDGSFFLYSRLTVDKSRWQEGNVFSCSVMHEALHNHYTQKSLSLSLGK

SEQ ID NO: 95 - protein, 107 aa, Artificial Sequence [sequence omitted]

SEQ ID NO: 96 - DNA, 15 bp, Artificial Sequence
tcctacggcatgcac

SEQ ID NO: 97 - DNA, 51 bp, Artificial Sequence
gtgatctgggaggatggctccaaccagtactatgccgacagcgtgaaggga

SEQ ID NO: 98 - DNA, 39 bp, Artificial Sequence
gacaaccaagacaccagccccgacgtgggcatcgattat

SEQ ID NO: 99 - DNA, 33 bp, Artificial Sequence
agagccagccagaacatctccccctttctgaat

SEQ ID NO: 100 - DNA, 21 bp, Artificial Sequence
gccgctgtgggactgcagagc

SEQ ID NO: 101 - DNA, 27 bp, Artificial Sequence
cagcagtataccgactaccctctgacc

SEQ ID NO: 102 - DNA, 366 bp, Artificial Sequence
caagtgcagctggtggagagcggaggaggagtggtgcaacccggcgagtccctcagactgagctgtgccgccagcggcttcaccttcagctcctacggcatgcactgggtgagacaagcccccggcaaaggactggagtgggtggccgtgatctgggaggatggctccaaccagtactatgccgacagcgtgaagggaagattcaccatctctagagacaactccaagaacacactgtatctgcagatgaactctctgagggccgaggacaccgccgtgtactactgcgccaaggacaaccaagacaccagccccgacgtgggcatcgattattggggccagggtaccctggttaccgttagcagc

SEQ ID NO: 103 - DNA, 321 bp, Artificial Sequence
gacatccagatgacccagagccctagctctctgtccgctagcgtgggagatagagtgaccatcacatgcagagccagccagaacatctccccctttctgaattggtatcagcagaagcccggcaaggcccctaagctgctgatctatgccgctgtgggactgcagagcggagtgccttccagattctccggcagcggcagcggaaccgacttcacactgaccatcagctctctgcagcccgaggacttcgccacctactactgccagcagtataccgactaccctctgaccttcggaggcggcaccaaggtggagatcaag

SEQ ID NO: 104 - protein, 8 aa, Artificial Sequence
GFTFSSYG

SEQ ID NO: 105 - DNA, 990 bp, Artificial Sequence
gcgagcaccaaaggcccgagcgtgtttccgctggccccgagcagcaaaagcaccagcggtggcaccgcagcgctgggttgcctggtgaaagattatttcccggaaccggtgacggtgtcgtggaactcaggcgccctgaccagcggcgtgcacaccttcccggctgtcctacagtcctcaggactctactccctcagcagcgtggtgaccgtgccctccagcagcttgggcacccagacctacatctgcaacgtgaatcacaagcccagcaacaccaaggtggacaagaaagttgagcccaaatcttgtgacaaaactcacacatgcccaccgtgcccagcacctgaactcctggggggaccgtcagtcttcctcttccccccaaaacccaaggacaccctcatgatctcccggacccctgaggtcacatgcgtggtggtggacgtgagccacgaagaccctgaggtcaagttcaactggtacgtggacggcgtggaggtgcataatgccaagacaaagccgcgggaggagcagtacaacagcacgtaccgtgtggtcagcgtcctcaccgtcctgcaccaggactggctgaatggcaaggagtacaagtgcaaggtctccaacaaagccctcccagcccccatcgagaaaaccatctccaaagccaaagggcagccccgagaaccacaggtgtacaccctgcccccatcccgggatgagctgaccaagaaccaggtcagcctgacctgcctggtcaaaggcttctatcccagcgacatcgccgtggagtgggagagcaatgggcagccggagaacaactacaagaccacgcctcccgtgctggactccgacggctccttcttcctctacagcaagctcaccgtggacaagagcaggtggcagcaggggaacgtcttctcatgctccgtgatgcatgaggctctgcacaaccactacacgcagaagagcctctccctgtctccgggtaaa

SEQ ID NO: 106 - DNA, 321 bp, Artificial Sequence
cgtacggtggctgcaccatctgtcttcatcttcccgccatctgatgagcagttgaaatctggaactgcctctgttgtgtgcctgctgaataacttctatcccagagaggccaaagtacagtggaaggtggataacgccctccaatcgggtaactcccaggagagtgtcacagagcaggacagcaaggacagcacctacagcctcagcagcaccctgacgctgagcaaagcagactacgagaaacacaaagtctacgcctgcgaagtcacccatcagggcctgagctcgcccgtcacaaagagcttcaacaggggagagtgt